European Patent Specification EP 3 706 773 B1, published August 26, 2026. Title: Maturation of mucosal defense and gut/lung function in the preterm infant. Applicant: Defensin Therapeutics ApS. The sequence listing filed with the application follows.

SEQUENCE LISTING (16 sequences)

SEQ ID NO: 1 - protein, 36 aa, Homo sapiens
DHYNCVSSGGQCLYSACPIFTKIQGTCYRGKAKCCK

SEQ ID NO: 2 - protein, 41 aa, Homo sapiens
GIGDPVTCLKSGAICHPVFCPRRYKQIGTCGLPGTKCCKKP

SEQ ID NO: 3 - protein, 44 aa, Homo sapiens
GIINTLQKYYCRVRGGRCAVLSCLPKEEQIGKCSTRGRKCCRRK

SEQ ID NO: 4 - protein, 37 aa, Homo sapiens
ELDRICGYGTARCRKKCRSQEYRIGRCPNTYACCLRK

SEQ ID NO: 5 - protein, 32 aa, Homo sapiens
ATCYCRTGRCATRESLSGVCEISGRLYRLCCR

SEQ ID NO: 6 - protein, 32 aa, Homo sapiens
AFTCHCRRSCYSTEYSYGTCTVMGINHRFCCL

SEQ ID NO: 7 - protein, 40 aa, Mus musculus
KINNPVSCLRKGGRCWNRCIGNTRQIGSCGVPFLKCCKRK

SEQ ID NO: 8 - protein, 30 aa, Homo sapiens
ACYCRIPACIAGERRYGTCIYQGRLWAFCC

SEQ ID NO: 9 - protein, 29 aa, Homo sapiens
CYCRIPACIAGERRYGTCIYQGRLWAFCC

SEQ ID NO: 10 - protein, 30 aa, Homo sapiens
DCYCRIPACIAGERRYGTCIYQGRLWAFCC

SEQ ID NO: 11 - protein, 33 aa, Homo sapiens
VCSCRLVFCRRTELRVGNCLIGGVSFTYCCTRV

SEQ ID NO: 12 - protein, 37 aa, Homo sapiens
LLGDFFRKSKEKIGKEFKRIVQRIKDFLRNLVPRTES

SEQ ID NO: 13 - protein, 690 aa, Homo sapiens
GRRRSVQWCAVSQPEATKCFQWQRNMRKVRGPPVSCIKRDSPIQCIQAIAENRADAVTLDGGFIYEAGLAPYKLRPVAAEVYGTERQPRTHYYAVAVVKKGGSFQLNELQGLKSCHTGLRRTAGWNVPIGTLRPFLNWTGPPEPIEAAVARFFSASCVPGADKGQFPNLCRLCAGTGENCAFSSQEPYFSYSGAFKCLRDGAGDVAFIRESTVFEDLSDEAERDEYELLCPDNTRKPVDKFKDCHLARVPSHAVVARSVNGKEDAIWNLLRQAQEKFGKDKSPKFQLFGSPSGQKDLLFKDSAIGFSRVPPRIDSGLYLGSGYFTAIQNLRKSEEEVAARRARVVWCAVGEQELRKCNQWSGLSEGSVTCSSASTTEDCIALVLKGEADAMSLDGGYVYTAGKCGLVPVLAENYKSQQSSDPDPNCVDRPVEGYLAVAVVRRSDTSLTWNSVKGKKSCHTAVDRTAGWNIPMGLLFNQTGSCKFDEYFSQSCAPGSDPRSNLCALCIGDEQGENKCVPNSNERYYGYTGAFRCLAENAGDVAFVKDVTVLQNTDGNNNEAWAKDLKLADFALLCLDGKRKPVTEARSCHLAMAPNHAVVSRMDKVERLKQVLLHQQAKFGRNGSDCPDKFCLFQSETKNLLFNDNTECLARLHGKTTYEKYLGPQYVAGITNLKKCSTSPLLEACEFLRK

SEQ ID NO: 14 - protein, 48 aa, Homo sapiens
GRRRSVQWCAVSQPEATKCFQWQRNMRKVRGPPVSCIKRDSPIQCIQA

SEQ ID NO: 15 - protein, 130 aa, Homo sapiens
KVFERCELARTLKRLGMDGYRGISLANWMCLAKWESGYNTRATNYNAGDRSTDYGIFQINSRYWCNDGKTPGAVNACHLSCSALLQDNIADAVACAKRVVRDPQGIRAWVAWRNRCQNRDVRQYVQGCGV

SEQ ID NO: 16 - protein, 37 aa, Homo sapiens
PVTCLKSGAICHPVFCPRRYKQIGTCGLPGTKCCKKP